European Patent Specification EP 3 931 191 B1, published October 4, 2023. Title: NOVEL COMPOUNDS AND PHARMACEUTICAL COMPOSITIONS THEREOF FOR THE TREATMENT OF DISEASES. Applicant: Galapagos NV. The sequence listing filed with the application follows.

SEQUENCE LISTING (2 sequences)

SEQ ID NO: 1 - DNA, 9428 bp, Artificial Sequence
  pcDNA3.1-PASK(FL,WT)-FLAG
gacggatcgggagatctcccgatcccctatggtgcactctcagtacaatctgctctgatgccgcatagttaagccagtatctgctccctgcttgtgtgttggaggtcgctgagtagtgcgcgagcaaaatttaagctacaacaaggcaaggcttgaccgacaattgcatgaagaatctgcttagggttaggcgttttgcgctgcttcgcgatgtacgggccagatatacgcgttgacattgattattgactagttattaatagtaatcaattacggggtcattagttcatagcccatatatggagttccgcgttacataacttacggtaaatggcccgcctggctgaccgcccaacgacccccgcccattgacgtcaataatgacgtatgttcccatagtaacgccaatagggactttccattgacgtcaatgggtggagtatttacggtaaactgcccacttggcagtacatcaagtgtatcatatgccaagtacgccccctattgacgtcaatgacggtaaatggcccgcctggcattatgcccagtacatgaccttatgggactttcctacttggcagtacatctacgtattagtcatcgctattaccatggtgatgcggttttggcagtacatcaatgggcgtggatagcggtttgactcacggggatttccaagtctccaccccattgacgtcaatgggagtttgttttggcaccaaaatcaacgggactttccaaaatgtcgtaacaactccgccccattgacgcaaatgggcggtaggcgtgtacggtgggaggtctatataagcagagctctctggctaactagagaacccactgcttactggcttatcgaaattaatacgactcactatagggagacccaagctggctagcgtttaaacttaagcttggtaccgagctcggatccactagtccagtgtggtggaattctgcagatatccagcacagtggcggccgcatggaggacgggggcttaacagcctttgaagaggaccagagatgcctttcccagagcctccccttgccagtgtcagcagagggcccagctgcacagaccactgctgagcccagcaggtcgttttcctcagcccacagacacctgagcagaaggaatgggctttccagactctgccagagcaggacagcgctctctgaagacagatggagctcctattgtctatcatcactggctgcccagaatatttgtacaagtaaactgcactgccctgctgcccctgagcacacggacccgtccgaaccgcggggcagtgtgtcctgctgctccctgctgcggggactgtcctcagggtggtcctcacctctgcttccggcccctgtgtgcaaccctaacaaggccatcttcacggtggatgccaagaccacagagatcctggttgctaacgacaaagcttgcgggctcctggggtacagcagccaggacctgattggccagaagctcacgcagttctttctgaggtcagattctgatgtggtggaggccctcagcgaggagcacatggaggccgacggccacgctgcggtggtgtttggcacggtggtggacatcatcagccgtagtggggagaagattccagtgtctgtgtggatgaagaggatgcggcaggagcgccgcctatgctgcgtggtggtcctggagcccgtggagagggtctcgacctgggtcgctttccagagcgatggcaccgtcacgtcatgtgacagtctctttgctcatcttcacgggtacgtgtctggggaggacgtggctgggcagcatatcacagacctgatcccttctgtgcagctccctccttctggccagcacatcccaaagaatctcaagattcagaggtctgttggaagagccagggacggtaccaccttccctctgagcttaaagctgaaatcccaacccagcagcgaggaggcgaccaccggtgaggcggcccctgtgagcggctaccgggcatctgtctgggtgttctgcaccatcagtggcctcatcaccctcctgccggatgggaccatccacggcatcaaccacagcttcgcgctgacactgtttggttacggaaagacggagctcctgggcaagaatatcactttcctgattcctggtttctacagctacatggaccttgcgtacaacagctcattacagctcccagacctggccagctgcctggacgtcggcaatgagagtgggtgtggggagagaaccttggacccgtggcagggccaggacccagctgaggggggccaggatccaaggattaatgtcgtgcttgctggtggccacgttgtgccccgagatgagatccggaagctgatggaaagccaagacatcttcaccgggactcagactgagctgattgctggaggccagctcctttcctgcctctcacctcagcctgctccaggggtggacaatgtcccagaaggaagcctgccagtgcacggtgaacaggcgctgcccaaggaccagcaaatcactgccttggggagagaggaacctgtggcaatagagagccccggacaggatcttctgggagaaagcaggtctgaaccagtggatgtgaagccatttgcttcctgcgaagattctgaagctccagtcccagctgaggatgggggcagtgatgctggcatgtgtggcctgtgtcagaaggcccagctagagcggatgggagtcagtggtcccagcggttcagacctttgggctggggctgccgtggccaagccccaggccaagggtcagctggcggggggcagcctcctgatgcactgcccttgctatgggagtgaatggggcttgtggtggcgaagccaggacttggcccccagcccctctgggatggcaggcctctcgtttgggacacctactctagatgagccgtggctgggagtggaaaacgaccgagaagagctgcagacctgcttgattaaggagcagctgtcccagttgagccttgcaggagccctggatgtcccccacgccgaactcgttccgacagagtgccaggctgtcaccgctcctgtgtcgtcctgcgatctgggaggcagagacctgtgcggtggctgcacgggcagctcctcagcctgctatgccttggccacggacctccctgggggcctggaagcagtggaggcccaggaggttgatgtgaattcgttttcctggaacctcaaggaactctttttcagtgaccagacagaccaaacgtcatcaaattgttcctgtgctacgtctgaactcagagagacaccctcttccttggcagtgggctccgatccagatgtaggcagtctccaggaacaggggtcgtgtgtcctggatgacagggagctgttactactgaccggcacctgtgttgaccttggccaaggccgacggttccgggagagctgtgtgggacatgatccaacagaaccgcttgaggtttgtttggtgtcctctgagcattatgcagcaagcgacagagaaagcccaggacacgttccttccacgttggatgctggccctgaggacacgtgcccatcagcagaggagccaaggctgaacgtccaggtcacctccacgcccgtgatcgtgatgcgcggggctgctggcctgcagcgggagatccaggagggtgcctactccgggagctgctaccatcgagatggcttacggctgagtatacagtttgaggtgaggcgggtggagctccagggccccacacctctgttctgctgctggctggtgaaagacctcctccacagccaacgcgactcagccgccaggacccgcctgttccttgccagcctgcccggctccacccactctaccgctgctgagctcaccggacccagcctggtggaagtgctcagagccagaccctggtttgaggagccccccaaggctgtggaactggaggggttggcggcctgtgagggcgagtactcccaaaagtacagtaccatgagcccgctgggcagtggggccttcggcttcgtgtggactgctgtggacaaggaaaaaaacaaggaggtggtggtgaagtttattaagaaggagaaggtcttggaggattgttggattgaggatcccaaacttgggaaagttactttagagatcgcaattctatccagggtggagcacgccaatatcatcaaggtattggatatatttgaaaaccaagggttcttccagcttgtgatggagaagcacggctccggcctagacctcttcgctttcatcgaccgccaccccaggctggatgagcccctggcgagctacatcttccgacaactagtgtcagcagtgggatacctgcgcttgaaggacatcatccaccgtgacatcaaggatgagaacatcgtgatcgccgaggacttcacaatcaagctgatagactttggctcggccgcctacttggaaaggggaaaattattttatactttttgtgggaccatcgagtactgtgcaccggaagttctcatggggaatccctacagagggccggagctggagatgtggtctctgggagtcactctgtacacgctggtctttgaggagaaccccttctgtgagctggaggagaccgtggaggctgccatacacccgccatacctggtgtccaaagaactcatgagccttgtgtctgggctgctgcagccagtccctgagagacgcaccaccttggagaagctggtgacagacccgtgggtaacacagcctgtgaatcttgctgactatacatgggaagaggtgtttcgagtaaacaagccagaaagtggagttctgtccgctgcgagcctggagatggggaacaggagcctgagtgatgtggcccaggctcaggagctttgtgggggccccgttccaggcgaggctcctaatggccaaggctgtttgcatcccggggatccccgtctgctgaccagcgattacaaggatgacgatgataagtagtgactcgagtctagagggcccgtttaaacccgctgatcagcctcgactgtgccttctagttgccagccatctgttgtttgcccctcccccgtgccttccttgaccctggaaggtgccactcccactgtcctttcctaataaaatgaggaaattgcatcgcattgtctgagtaggtgtcattctattctggggggtggggtggggcaggacagcaagggggaggattgggaagacaatagcaggcatgctggggatgcggtgggctctatggcttctgaggcggaaagaaccagctggggctctagggggtatccccacgcgccctgtagcggcgcattaagcgcggcgggtgtggtggttacgcgcagcgtgaccgctacacttgccagcgccctagcgcccgctcctttcgctttcttcccttcctttctcgccacgttcgccggctttccccgtcaagctctaaatcgggggctccctttagggttccgatttagtgctttacggcacctcgaccccaaaaaacttgattagggtgatggttcacgtagtgggccatcgccctgatagacggtttttcgccctttgacgttggagtccacgttctttaatagtggactcttgttccaaactggaacaacactcaaccctatctcggtctattcttttgatttataagggattttgccgatttcggcctattggttaaaaaatgagctgatttaacaaaaatttaacgcgaattaattctgtggaatgtgtgtcagttagggtgtggaaagtccccaggctccccagcaggcagaagtatgcaaagcatgcatctcaattagtcagcaaccaggtgtggaaagtccccaggctccccagcaggcagaagtatgcaaagcatgcatctcaattagtcagcaaccatagtcccgcccctaactccgcccatcccgcccctaactccgcccagttccgcccattctccgccccatggctgactaattttttttatttatgcagaggccgaggccgcctctgcctctgagctattccagaagtagtgaggaggcttttttggaggcctaggcttttgcaaaaagctcccgggagcttgtatatccattttcggatctgatcaagagacaggatgaggatcgtttcgcatgattgaacaagatggattgcacgcaggttctccggccgcttgggtggagaggctattcggctatgactgggcacaacagacaatcggctgctctgatgccgccgtgttccggctgtcagcgcaggggcgcccggttctttttgtcaagaccgacctgtccggtgccctgaatgaactgcaggacgaggcagcgcggctatcgtggctggccacgacgggcgttccttgcgcagctgtgctcgacgttgtcactgaagcgggaagggactggctgctattgggcgaagtgccggggcaggatctcctgtcatctcaccttgctcctgccgagaaagtatccatcatggctgatgcaatgcggcggctgcatacgcttgatccggctacctgcccattcgaccaccaagcgaaacatcgcatcgagcgagcacgtactcggatggaagccggtcttgtcgatcaggatgatctggacgaagagcatcaggggctcgcgccagccgaactgttcgccaggctcaaggcgcgcatgcccgacggcgaggatctcgtcgtgacccatggcgatgcctgcttgccgaatatcatggtggaaaatggccgcttttctggattcatcgactgtggccggctgggtgtggcggaccgctatcaggacatagcgttggctacccgtgatattgctgaagagcttggcggcgaatgggctgaccgcttcctcgtgctttacggtatcgccgctcccgattcgcagcgcatcgccttctatcgccttcttgacgagttcttctgagcgggactctggggttcgaaatgaccgaccaagcgacgcccaacctgccatcacgagatttcgattccaccgccgccttctatgaaaggttgggcttcggaatcgttttccgggacgccggctggatgatcctccagcgcggggatctcatgctggagttcttcgcccaccccaacttgtttattgcagcttataatggttacaaataaagcaatagcatcacaaatttcacaaataaagcatttttttcactgcattctagttgtggtttgtccaaactcatcaatgtatcttatcatgtctgtataccgtcgacctctagctagagcttggcgtaatcatggtcatagctgtttcctgtgtgaaattgttatccgctcacaattccacacaacatacgagccggaagcataaagtgtaaagcctggggtgcctaatgagtgagctaactcacattaattgcgttgcgctcactgcccgctttccagtcgggaaacctgtcgtgccagctgcattaatgaatcggccaacgcgcggggagaggcggtttgcgtattgggcgctcttccgcttcctcgctcactgactcgctgcgctcggtcgttcggctgcggcgagcggtatcagctcactcaaaggcggtaatacggttatccacagaatcaggggataacgcaggaaagaacatgtgagcaaaaggccagcaaaaggccaggaaccgtaaaaaggccgcgttgctggcgtttttccataggctccgcccccctgacgagcatcacaaaaatcgacgctcaagtcagaggtggcgaaacccgacaggactataaagataccaggcgtttccccctggaagctccctcgtgcgctctcctgttccgaccctgccgcttaccggatacctgtccgcctttctcccttcgggaagcgtggcgctttctcatagctcacgctgtaggtatctcagttcggtgtaggtcgttcgctccaagctgggctgtgtgcacgaaccccccgttcagcccgaccgctgcgccttatccggtaactatcgtcttgagtccaacccggtaagacacgacttatcgccactggcagcagccactggtaacaggattagcagagcgaggtatgtaggcggtgctacagagttcttgaagtggtggcctaactacggctacactagaagaacagtatttggtatctgcgctctgctgaagccagttaccttcggaaaaagagttggtagctcttgatccggcaaacaaaccaccgctggtagcggtttttttgtttgcaagcagcagattacgcgcagaaaaaaaggatctcaagaagatcctttgatcttttctacggggtctgacgctcagtggaacgaaaactcacgttaagggattttggtcatgagattatcaaaaaggatcttcacctagatccttttaaattaaaaatgaagttttaaatcaatctaaagtatatatgagtaaacttggtctgacagttaccaatgcttaatcagtgaggcacctatctcagcgatctgtctatttcgttcatccatagttgcctgactccccgtcgtgtagataactacgatacgggagggcttaccatctggccccagtgctgcaatgataccgcgagacccacgctcaccggctccagatttatcagcaataaaccagccagccggaagggccgagcgcagaagtggtcctgcaactttatccgcctccatccagtctattaattgttgccgggaagctagagtaagtagttcgccagttaatagtttgcgcaacgttgttgccattgctacaggcatcgtggtgtcacgctcgtcgtttggtatggcttcattcagctccggttcccaacgatcaaggcgagttacatgatcccccatgttgtgcaaaaaagcggttagctccttcggtcctccgatcgttgtcagaagtaagttggccgcagtgttatcactcatggttatggcagcactgcataattctcttactgtcatgccatccgtaagatgcttttctgtgactggtgagtactcaaccaagtcattctgagaatagtgtatgcggcgaccgagttgctcttgcccggcgtcaatacgggataataccgcgccacatagcagaactttaaaagtgctcatcattggaaaacgttcttcggggcgaaaactctcaaggatcttaccgctgttgagatccagttcgatgtaacccactcgtgcacccaactgatcttcagcatcttttactttcaccagcgtttctgggtgagcaaaaacaggaaggcaaaatgccgcaaaaaagggaataagggcgacacggaaatgttgaatactcatactcttcctttttcaatattattgaagcatttatcagggttattgtctcatgagcggatacatatttgaatgtatttagaaaaataaacaaataggggttccgcgcacatttccccgaaaagtgccacctgacgtc

SEQ ID NO: 2 - DNA, 9428 bp, Artificial Sequence
  pcDNA3.1-PASK(FL,DN)-FLAG
gacggatcgggagatctcccgatcccctatggtgcactctcagtacaatctgctctgatgccgcatagttaagccagtatctgctccctgcttgtgtgttggaggtcgctgagtagtgcgcgagcaaaatttaagctacaacaaggcaaggcttgaccgacaattgcatgaagaatctgcttagggttaggcgttttgcgctgcttcgcgatgtacgggccagatatacgcgttgacattgattattgactagttattaatagtaatcaattacggggtcattagttcatagcccatatatggagttccgcgttacataacttacggtaaatggcccgcctggctgaccgcccaacgacccccgcccattgacgtcaataatgacgtatgttcccatagtaacgccaatagggactttccattgacgtcaatgggtggagtatttacggtaaactgcccacttggcagtacatcaagtgtatcatatgccaagtacgccccctattgacgtcaatgacggtaaatggcccgcctggcattatgcccagtacatgaccttatgggactttcctacttggcagtacatctacgtattagtcatcgctattaccatggtgatgcggttttggcagtacatcaatgggcgtggatagcggtttgactcacggggatttccaagtctccaccccattgacgtcaatgggagtttgttttggcaccaaaatcaacgggactttccaaaatgtcgtaacaactccgccccattgacgcaaatgggcggtaggcgtgtacggtgggaggtctatataagcagagctctctggctaactagagaacccactgcttactggcttatcgaaattaatacgactcactatagggagacccaagctggctagcgtttaaacttaagcttggtaccgagctcggatccactagtccagtgtggtggaattctgcagatatccagcacagtggcggccgcatggaggacgggggcttaacagcctttgaagaggaccagagatgcctttcccagagcctccccttgccagtgtcagcagagggcccagctgcacagaccactgctgagcccagcaggtcgttttcctcagcccacagacacctgagcagaaggaatgggctttccagactctgccagagcaggacagcgctctctgaagacagatggagctcctattgtctatcatcactggctgcccagaatatttgtacaagtaaactgcactgccctgctgcccctgagcacacggacccgtccgaaccgcggggcagtgtgtcctgctgctccctgctgcggggactgtcctcagggtggtcctcacctctgcttccggcccctgtgtgcaaccctaacaaggccatcttcacggtggatgccaagaccacagagatcctggttgctaacgacaaagcttgcgggctcctggggtacagcagccaggacctgattggccagaagctcacgcagttctttctgaggtcagattctgatgtggtggaggccctcagcgaggagcacatggaggccgacggccacgctgcggtggtgtttggcacggtggtggacatcatcagccgtagtggggagaagattccagtgtctgtgtggatgaagaggatgcggcaggagcgccgcctatgctgcgtggtggtcctggagcccgtggagagggtctcgacctgggtcgctttccagagcgatggcaccgtcacgtcatgtgacagtctctttgctcatcttcacgggtacgtgtctggggaggacgtggctgggcagcatatcacagacctgatcccttctgtgcagctccctccttctggccagcacatcccaaagaatctcaagattcagaggtctgttggaagagccagggacggtaccaccttccctctgagcttaaagctgaaatcccaacccagcagcgaggaggcgaccaccggtgaggcggcccctgtgagcggctaccgggcatctgtctgggtgttctgcaccatcagtggcctcatcaccctcctgccggatgggaccatccacggcatcaaccacagcttcgcgctgacactgtttggttacggaaagacggagctcctgggcaagaatatcactttcctgattcctggtttctacagctacatggaccttgcgtacaacagctcattacagctcccagacctggccagctgcctggacgtcggcaatgagagtgggtgtggggagagaaccttggacccgtggcagggccaggacccagctgaggggggccaggatccaaggattaatgtcgtgcttgctggtggccacgttgtgccccgagatgagatccggaagctgatggaaagccaagacatcttcaccgggactcagactgagctgattgctggaggccagctcctttcctgcctctcacctcagcctgctccaggggtggacaatgtcccagaaggaagcctgccagtgcacggtgaacaggcgctgcccaaggaccagcaaatcactgccttggggagagaggaacctgtggcaatagagagccccggacaggatcttctgggagaaagcaggtctgaaccagtggatgtgaagccatttgcttcctgcgaagattctgaagctccagtcccagctgaggatgggggcagtgatgctggcatgtgtggcctgtgtcagaaggcccagctagagcggatgggagtcagtggtcccagcggttcagacctttgggctggggctgccgtggccaagccccaggccaagggtcagctggcggggggcagcctcctgatgcactgcccttgctatgggagtgaatggggcttgtggtggcgaagccaggacttggcccccagcccctctgggatggcaggcctctcgtttgggacacctactctagatgagccgtggctgggagtggaaaacgaccgagaagagctgcagacctgcttgattaaggagcagctgtcccagttgagccttgcaggagccctggatgtcccccacgccgaactcgttccgacagagtgccaggctgtcaccgctcctgtgtcgtcctgcgatctgggaggcagagacctgtgcggtggctgcacgggcagctcctcagcctgctatgccttggccacggacctccctgggggcctggaagcagtggaggcccaggaggttgatgtgaattcgttttcctggaacctcaaggaactctttttcagtgaccagacagaccaaacgtcatcaaattgttcctgtgctacgtctgaactcagagagacaccctcttccttggcagtgggctccgatccagatgtaggcagtctccaggaacaggggtcgtgtgtcctggatgacagggagctgttactactgaccggcacctgtgttgaccttggccaaggccgacggttccgggagagctgtgtgggacatgatccaacagaaccgcttgaggtttgtttggtgtcctctgagcattatgcagcaagcgacagagaaagcccaggacacgttccttccacgttggatgctggccctgaggacacgtgcccatcagcagaggagccaaggctgaacgtccaggtcacctccacgcccgtgatcgtgatgcgcggggctgctggcctgcagcgggagatccaggagggtgcctactccgggagctgctaccatcgagatggcttacggctgagtatacagtttgaggtgaggcgggtggagctccagggccccacacctctgttctgctgctggctggtgaaagacctcctccacagccaacgcgactcagccgccaggacccgcctgttccttgccagcctgcccggctccacccactctaccgctgctgagctcaccggacccagcctggtggaagtgctcagagccagaccctggtttgaggagccccccaaggctgtggaactggaggggttggcggcctgtgagggcgagtactcccaaaagtacagtaccatgagcccgctgggcagtggggccttcggcttcgtgtggactgctgtggacaaggaaaaaaacaaggaggtggtggtgaggtttattaagaaggagaaggtcttggaggattgttggattgaggatcccaaacttgggaaagttactttagagatcgcaattctatccagggtggagcacgccaatatcatcaaggtattggatatatttgaaaaccaagggttcttccagcttgtgatggagaagcacggctccggcctagacctcttcgctttcatcgaccgccaccccaggctggatgagcccctggcgagctacatcttccgacaactagtgtcagcagtgggatacctgcgcttgaaggacatcatccaccgtgacatcaaggatgagaacatcgtgatcgccgaggacttcacaatcaagctgatagactttggctcggccgcctacttggaaaggggaaaattattttatactttttgtgggaccatcgagtactgtgcaccggaagttctcatggggaatccctacagagggccggagctggagatgtggtctctgggagtcactctgtacacgctggtctttgaggagaaccccttctgtgagctggaggagaccgtggaggctgccatacacccgccatacctggtgtccaaagaactcatgagccttgtgtctgggctgctgcagccagtccctgagagacgcaccaccttggagaagctggtgacagacccgtgggtaacacagcctgtgaatcttgctgactatacatgggaagaggtgtttcgagtaaacaagccagaaagtggagttctgtccgctgcgagcctggagatggggaacaggagcctgagtgatgtggcccaggctcaggagctttgtgggggccccgttccaggcgaggctcctaatggccaaggctgtttgcatcccggggatccccgtctgctgaccagcgattacaaggatgacgatgataagtagtgactcgagtctagagggcccgtttaaacccgctgatcagcctcgactgtgccttctagttgccagccatctgttgtttgcccctcccccgtgccttccttgaccctggaaggtgccactcccactgtcctttcctaataaaatgaggaaattgcatcgcattgtctgagtaggtgtcattctattctggggggtggggtggggcaggacagcaagggggaggattgggaagacaatagcaggcatgctggggatgcggtgggctctatggcttctgaggcggaaagaaccagctggggctctagggggtatccccacgcgccctgtagcggcgcattaagcgcggcgggtgtggtggttacgcgcagcgtgaccgctacacttgccagcgccctagcgcccgctcctttcgctttcttcccttcctttctcgccacgttcgccggctttccccgtcaagctctaaatcgggggctccctttagggttccgatttagtgctttacggcacctcgaccccaaaaaacttgattagggtgatggttcacgtagtgggccatcgccctgatagacggtttttcgccctttgacgttggagtccacgttctttaatagtggactcttgttccaaactggaacaacactcaaccctatctcggtctattcttttgatttataagggattttgccgatttcggcctattggttaaaaaatgagctgatttaacaaaaatttaacgcgaattaattctgtggaatgtgtgtcagttagggtgtggaaagtccccaggctccccagcaggcagaagtatgcaaagcatgcatctcaattagtcagcaaccaggtgtggaaagtccccaggctccccagcaggcagaagtatgcaaagcatgcatctcaattagtcagcaaccatagtcccgcccctaactccgcccatcccgcccctaactccgcccagttccgcccattctccgccccatggctgactaattttttttatttatgcagaggccgaggccgcctctgcctctgagctattccagaagtagtgaggaggcttttttggaggcctaggcttttgcaaaaagctcccgggagcttgtatatccattttcggatctgatcaagagacaggatgaggatcgtttcgcatgattgaacaagatggattgcacgcaggttctccggccgcttgggtggagaggctattcggctatgactgggcacaacagacaatcggctgctctgatgccgccgtgttccggctgtcagcgcaggggcgcccggttctttttgtcaagaccgacctgtccggtgccctgaatgaactgcaggacgaggcagcgcggctatcgtggctggccacgacgggcgttccttgcgcagctgtgctcgacgttgtcactgaagcgggaagggactggctgctattgggcgaagtgccggggcaggatctcctgtcatctcaccttgctcctgccgagaaagtatccatcatggctgatgcaatgcggcggctgcatacgcttgatccggctacctgcccattcgaccaccaagcgaaacatcgcatcgagcgagcacgtactcggatggaagccggtcttgtcgatcaggatgatctggacgaagagcatcaggggctcgcgccagccgaactgttcgccaggctcaaggcgcgcatgcccgacggcgaggatctcgtcgtgacccatggcgatgcctgcttgccgaatatcatggtggaaaatggccgcttttctggattcatcgactgtggccggctgggtgtggcggaccgctatcaggacatagcgttggctacccgtgatattgctgaagagcttggcggcgaatgggctgaccgcttcctcgtgctttacggtatcgccgctcccgattcgcagcgcatcgccttctatcgccttcttgacgagttcttctgagcgggactctggggttcgaaatgaccgaccaagcgacgcccaacctgccatcacgagatttcgattccaccgccgccttctatgaaaggttgggcttcggaatcgttttccgggacgccggctggatgatcctccagcgcggggatctcatgctggagttcttcgcccaccccaacttgtttattgcagcttataatggttacaaataaagcaatagcatcacaaatttcacaaataaagcatttttttcactgcattctagttgtggtttgtccaaactcatcaatgtatcttatcatgtctgtataccgtcgacctctagctagagcttggcgtaatcatggtcatagctgtttcctgtgtgaaattgttatccgctcacaattccacacaacatacgagccggaagcataaagtgtaaagcctggggtgcctaatgagtgagctaactcacattaattgcgttgcgctcactgcccgctttccagtcgggaaacctgtcgtgccagctgcattaatgaatcggccaacgcgcggggagaggcggtttgcgtattgggcgctcttccgcttcctcgctcactgactcgctgcgctcggtcgttcggctgcggcgagcggtatcagctcactcaaaggcggtaatacggttatccacagaatcaggggataacgcaggaaagaacatgtgagcaaaaggccagcaaaaggccaggaaccgtaaaaaggccgcgttgctggcgtttttccataggctccgcccccctgacgagcatcacaaaaatcgacgctcaagtcagaggtggcgaaacccgacaggactataaagataccaggcgtttccccctggaagctccctcgtgcgctctcctgttccgaccctgccgcttaccggatacctgtccgcctttctcccttcgggaagcgtggcgctttctcatagctcacgctgtaggtatctcagttcggtgtaggtcgttcgctccaagctgggctgtgtgcacgaaccccccgttcagcccgaccgctgcgccttatccggtaactatcgtcttgagtccaacccggtaagacacgacttatcgccactggcagcagccactggtaacaggattagcagagcgaggtatgtaggcggtgctacagagttcttgaagtggtggcctaactacggctacactagaagaacagtatttggtatctgcgctctgctgaagccagttaccttcggaaaaagagttggtagctcttgatccggcaaacaaaccaccgctggtagcggtttttttgtttgcaagcagcagattacgcgcagaaaaaaaggatctcaagaagatcctttgatcttttctacggggtctgacgctcagtggaacgaaaactcacgttaagggattttggtcatgagattatcaaaaaggatcttcacctagatccttttaaattaaaaatgaagttttaaatcaatctaaagtatatatgagtaaacttggtctgacagttaccaatgcttaatcagtgaggcacctatctcagcgatctgtctatttcgttcatccatagttgcctgactccccgtcgtgtagataactacgatacgggagggcttaccatctggccccagtgctgcaatgataccgcgagacccacgctcaccggctccagatttatcagcaataaaccagccagccggaagggccgagcgcagaagtggtcctgcaactttatccgcctccatccagtctattaattgttgccgggaagctagagtaagtagttcgccagttaatagtttgcgcaacgttgttgccattgctacaggcatcgtggtgtcacgctcgtcgtttggtatggcttcattcagctccggttcccaacgatcaaggcgagttacatgatcccccatgttgtgcaaaaaagcggttagctccttcggtcctccgatcgttgtcagaagtaagttggccgcagtgttatcactcatggttatggcagcactgcataattctcttactgtcatgccatccgtaagatgcttttctgtgactggtgagtactcaaccaagtcattctgagaatagtgtatgcggcgaccgagttgctcttgcccggcgtcaatacgggataataccgcgccacatagcagaactttaaaagtgctcatcattggaaaacgttcttcggggcgaaaactctcaaggatcttaccgctgttgagatccagttcgatgtaacccactcgtgcacccaactgatcttcagcatcttttactttcaccagcgtttctgggtgagcaaaaacaggaaggcaaaatgccgcaaaaaagggaataagggcgacacggaaatgttgaatactcatactcttcctttttcaatattattgaagcatttatcagggttattgtctcatgagcggatacatatttgaatgtatttagaaaaataaacaaataggggttccgcgcacatttccccgaaaagtgccacctgacgtc